European Patent Application EP 4 566 617 A2, published June 11, 2025. Title: PEPTIDE COMPOUNDS AND THERAPEUTIC USES OF SAME. Applicant: Immunity Pharma Ltd. The sequence listing filed with the application follows.

SEQUENCE LISTING (21 sequences)

SEQ ID NO: 1 - skipped

SEQ ID NO: 2 - protein, 7 aa, synthetic construct
  REGION 1..7: note = Stressin-1 amino acid sequence
LPPLPYP

SEQ ID NO: 3 - protein, 5 aa, synthetic construct
  REGION 1..5: note = Synthetic Peptide
PPLPY

SEQ ID NO: 4 - protein, 7 aa, synthetic construct
  REGION 1..7: note = Synthetic Peptide
LPPLAYP

SEQ ID NO: 5-6 - skipped (2 entries)

SEQ ID NO: 7 - protein, 6 aa, synthetic construct
  REGION 1..6: note = Synthetic Peptide
LPPLPY

SEQ ID NO: 8 - protein, 6 aa, synthetic construct
  REGION 1..6: note = Synthetic Peptide
PPLPYP

SEQ ID NO: 9 - protein, 5 aa, synthetic construct
  REGION 1..5: note = Synthetic Peptide
PLPYP

SEQ ID NO: 10-12 - skipped (3 entries)

SEQ ID NO: 13 - protein, 7 aa, synthetic construct
  REGION 1..7: note = Synthetic Peptide
LPGLPYP

SEQ ID NO: 14 - protein, 7 aa, synthetic construct
  REGION 1..7: note = Synthetic Peptide
LPPLGYP

SEQ ID NO: 15 - protein, 7 aa, synthetic construct
  REGION 1..7: note = Synthetic Peptide
LAPLPYP

SEQ ID NO: 16 - protein, 7 aa, synthetic construct
  REGION 1..7: note = Synthetic Peptide
LPALPYP

SEQ ID NO: 17 - skipped

SEQ ID NO: 18 - protein, 6 aa, synthetic construct
  REGION 1..6: note = Synthetic Peptide
PPLAYP

SEQ ID NO: 19 - protein, 5 aa, synthetic construct
  REGION 1..5: note = Synthetic Peptide
  MOD_RES 5: note = AMIDATION
PPLPY

SEQ ID NO: 20 - protein, 6 aa, synthetic construct
  REGION 1..6: note = Synthetic Peptide
  MOD_RES 1: note = may be D amino acid
  MOD_RES 3: note = may be D amino acid
LPPLPY

SEQ ID NO: 21 - protein, 7 aa, synthetic construct
  REGION 1..7: note = Synthetic Peptide
  MOD_RES 1: note = may be D amino acid
  MOD_RES 3: note = may be D amino acid
  MOD_RES 5: note = may be D amino acid
LPPLAYP